European Patent Application EP 4 524 158 A1, published March 19, 2025. Title: ANTIBODIES SPECIFICALLY RECOGNIZING GDF15 AND USES THEREOF. Applicant: STAIDSON (BEIJING) BIOPHARMACEUTICALS CO., LTD. The sequence listing filed with the application follows.

SEQUENCE LISTING (91 sequences)

SEQ ID NO: 1 - protein, 5 aa, synthetic construct
NYYMS

SEQ ID NO: 2 - protein, 5 aa, synthetic construct
DYYMT

SEQ ID NO: 3 - protein, 5 aa, synthetic construct
DYYMS

SEQ ID NO: 4 - protein, 5 aa, synthetic construct
SHWMS

SEQ ID NO: 5 - protein, 5 aa, synthetic construct
TYWMS

SEQ ID NO: 6 - protein, 5 aa, synthetic construct
SYDMT

SEQ ID NO: 7 - protein, 15 aa, synthetic construct
MISFSGTTYATWAKG

SEQ ID NO: 8 - protein, 15 aa, synthetic construct
MISFSGTTHATWAKG

SEQ ID NO: 9 - protein, 17 aa, synthetic construct
DIYGGSGTTDYASWVKG

SEQ ID NO: 10 - protein, 16 aa, synthetic construct
FVSPSGRAYYTSWVNG

SEQ ID NO: 11 - protein, 17 aa, synthetic construct
TIYAGSGGTWYASWVKG

SEQ ID NO: 12 - protein, 16 aa, synthetic construct
IINNSGNTYYASWAKG

SEQ ID NO: 13 - protein, 12 aa, synthetic construct
VVYAGWTYPLGI

SEQ ID NO: 14 - protein, 6 aa, synthetic construct
GITADI

SEQ ID NO: 15 - protein, 8 aa, synthetic construct
GYTSGLDI

SEQ ID NO: 16 - protein, 8 aa, synthetic construct
GPNYSDAI

SEQ ID NO: 17 - protein, 13 aa, synthetic construct
GILVYADYGDHNL

SEQ ID NO: 18 - protein, 11 aa, synthetic construct
QASQSISSVLS

SEQ ID NO: 19 - protein, 11 aa, synthetic construct
QASQSISSYLA

SEQ ID NO: 20 - protein, 13 aa, synthetic construct
QSSKSVVNGDWLA

SEQ ID NO: 21 - protein, 11 aa, synthetic construct
QASEYIYSSLA

SEQ ID NO: 22 - protein, 11 aa, synthetic construct
QASEDIYTNLA

SEQ ID NO: 23 - protein, 7 aa, synthetic construct
EASILAS

SEQ ID NO: 24 - protein, 7 aa, synthetic construct
EASTQAS

SEQ ID NO: 25 - protein, 7 aa, synthetic construct
EASTLAS

SEQ ID NO: 26 - protein, 7 aa, synthetic construct
KASTLAS

SEQ ID NO: 27 - protein, 7 aa, synthetic construct
DAATLAS

SEQ ID NO: 28 - protein, 7 aa, synthetic construct
DASDLAS

SEQ ID NO: 29 - protein, 7 aa, synthetic construct
AASTLAS

SEQ ID NO: 30 - protein, 12 aa, synthetic construct
QANYDVYNYGNP

SEQ ID NO: 31 - protein, 11 aa, synthetic construct
RCIYGDSYGAA

SEQ ID NO: 32 - protein, 11 aa, synthetic construct
AGVYNNDSDNG

SEQ ID NO: 33 - protein, 12 aa, synthetic construct
QCTDLSSSAGNT

SEQ ID NO: 34 - protein, 12 aa, synthetic construct
LGVYTYISADGA

SEQ ID NO: 35 - skipped

SEQ ID NO: 36 - protein, 15 aa, synthetic construct
  VARIANT 9: note = X is H or Y
MISFSGTTXATWAKG

SEQ ID NO: 37 - protein, 7 aa, synthetic construct
  VARIANT 4: note = X is I or T
  VARIANT 5: note = X is L or Q
EASXXAS

SEQ ID NO: 38 - protein, 116 aa, synthetic construct
QQLKESGGRLVTPGTPLTLTCTASGFSLSNYYMSWVRQAPGEGLEWIGMISFSGTTYATWAKGRFTISKTSTTVDLKITSPTTEDTATYFCARVVYAGWTYPLGIWGPGTLVTISS

SEQ ID NO: 39 - protein, 119 aa, synthetic construct
EVQLVESGGGLVKPGGSLRLSCAASGFSLSNYYMSWVRQAPGKGLEWIGMISFSGTTYATWAKGRFTISKDSSKNTVYLQINSLKTEDTAVYFCARVVYAGWTYPLGIWGQGTLVTVSS

SEQ ID NO: 40 - protein, 117 aa, synthetic construct
EVQLVESGGGLVKPGGSLRLSCAASGFSLSNYYMSWVRQAPGKGLEWIGMISFSGTTYATWAKGRFTISKDSSTVYLQINSLKTEDTAVYFCARVVYAGWTYPLGIWGQGTLVTVSS

SEQ ID NO: 41 - protein, 119 aa, synthetic construct
EVQLVESGGGLVKPGGSLRLSCAASGFSLSNYYMSWVRQAPGKGLEWIGMISFSGTTYATWAKGRFTISKDDSKNTVYLQINSLKTEDTAVYFCARVVYAGWTYPLGIWGQGTLVTVSS

SEQ ID NO: 42 - protein, 119 aa, synthetic construct
EVQLVESGGGLVKPGGSLRLSCAASGFSLSNYYMSWVRQAPGKGLEWIGMISFSGTTYATWAKGRFTISRDDSKNTVYLQINSLKTEDTAVYFCARVVYAGWTYPLGIWGQGTLVTVSS

SEQ ID NO: 43 - protein, 119 aa, synthetic construct
EVQLVESGGGLVKPGGSLRLSCAASGFSLSNYYMSWVRQAPGKGLEWVGMISFSGTTYATWAKGRFTISRDDSKNTVYLQINSLKTEDTAVYFCARVVYAGWTYPLGIWGQGTLVTVSS

SEQ ID NO: 44 - protein, 119 aa, synthetic construct
EVQLVESGGGLVKPGGSLRLSCAASGFSLSNYYMSWVRQAPGKGLEWVGMISFSGTTYATWAKGRFTISRDDSKNTLYLQMNSLKTEDTAVYFCARVVYAGWTYPLGIWGQGTLVTVSS

SEQ ID NO: 45 - protein, 116 aa, synthetic construct
QSLEESGGRLVTPGTPLTLTCTASGFSLSNYYMSWVRQAPGEGLEWIGMISFSGTTYATWAKGRFTISKTSTTVDLKITSPTTEDTATYFCARVVYAGWTYPLGIWGPGTLVTVSS

SEQ ID NO: 46 - protein, 116 aa, synthetic construct
QSVKESGGRLVTPGTPLTLTCTASGFSLSDYYMTWVRQAPGEGLEWIGMISFSGTTYATWAKGRFTISKASTTVDLKITSPTTEDTATYFCARVVYAGWTYPLGIWGPGTLVTVSS

SEQ ID NO: 47 - protein, 117 aa, synthetic construct
SQTVKESGGRLVTPGTPLTLTCTASGFSLSNYYMSWVRQAPGEGLEWIGMISFSGTTHATWAKGRFTISKTSTTVDLKITSPTSEDTATYFCARVVYAGWTYPLGIWGPGTLVTVSS

SEQ ID NO: 48 - protein, 112 aa, synthetic construct
QQLKESGGRLVTPGTPLTLTCTVSGFSLSDYYMSWVRQAPGKGLEWIGDIYGGSGTTDYASWVKGRFTISKTSTTVDLRIASPTTEDTATYFCGRGITADIWGPGTLVTVSL

SEQ ID NO: 49 - protein, 113 aa, synthetic construct
QSVKESEGRLVTPGTPLTLTCTASGFSLSSHWMSWVRQAPGKGLEWIGFVSPSGRAYYTSWVNGRFTISKTSTTVDLKITSPTTEDTATYFCARGYTSGLDIWGPGTLVTVSS

SEQ ID NO: 50 - protein, 114 aa, synthetic construct
QSVKESGGRLVTPGTPLTLTCKASGFSLSTYWMSWVRQAPGKGLEWIGTIYAGSGGTWYASWVKGRFTISKTSTTVDLKMTSLTTEDTATYFCVRGPNYSDAIWGPGTLVTVSS

SEQ ID NO: 51 - protein, 118 aa, synthetic construct
QQLKESGGRLVTPGTPLTLTCTVSGFSLSSYDMTWVRQVPGKGLEWIGIINNSGNTYYASWAKGRFTISKTSTTVDLKITSPTTEDTATYFCARGILVYADYGDHNLWGPGTLVTVSS

SEQ ID NO: 52 - protein, 110 aa, synthetic construct
AVVLTQTAASVSEPVGGTVTIKCQASQSISSVLSWYQQKPGQPPKALIYEASILASGVPSRFKGSGSGTDFTLTISDLECADAATYYCQANYDVYNYGNPFGGGTEVVVK

SEQ ID NO: 53 - protein, 110 aa, synthetic construct
DIQLTQSPSSLSASVGDRVTITCQASQSISSVLSWYQQKPGKPPKALIYEASILASGVPSRFSGSGSGTDFTLTISSLQPEDFATYYCQANYDVYNYGNPFGGGTKVEIK

SEQ ID NO: 54 - protein, 110 aa, synthetic construct
DIQMTQSPSSLSASVGDRVTITCQASQSISSVLSWYQQKPGKPPKALIYEASILASGVPSRFSGSGSGTDFTLTISSLQPEDFATYYCQANYDVYNYGNPFGGGTKVEIK

SEQ ID NO: 55 - protein, 110 aa, synthetic construct
DIQMTQSPSSLSASVGDRVTITCQASQSISSVLSWYQQKPGKPPKLLIYEASILASGVPSRFSGSGSGTDFTLTISSLQPEDFATYYCQANYDVYNYGNPFGGGTKVEIK

SEQ ID NO: 56 - protein, 110 aa, synthetic construct
AINMTQTPASVSEPVGGTVTIKCQASQSISSVLSWYQQKPGQPPKVLIYEASTQASGVPSRFKGSGSGTDFTLTISDLECADAATYYCQANYDVYNYGNPFGGGTEVVVK

SEQ ID NO: 57 - protein, 110 aa, synthetic construct
DPVLTQTPASVSEPVGGTVTIKCQASQSISSVLSWYQQKPGQPPKVLIYEASTLASGVPSRFKGSGSGTDFTLTISDLECADAATYYCQANYDVYNYGNPFGGGTEVVVK

SEQ ID NO: 58 - protein, 110 aa, synthetic construct
YVMMTQTPPSVSEPVGGTVTIKCQASQSISSVLSWYQQKPGQPPKVLIYEASTLASGVPSRFKGSGSGTDFTLTISDLECADAATYYCQANYDVYNYGNPFGGGTEVVVK

SEQ ID NO: 59 - protein, 110 aa, synthetic construct
AQVMTQTPASVSEPVGGTVTIKCQASQSISSVLSWYQQKPGQPPKVLIYEASTLASGVPSRFKGSGSGTDFTLAISDLECADAATYYCQANYDVYNYGNPFGGGTEVVVK

SEQ ID NO: 60 - protein, 109 aa, synthetic construct
DIVLTQTPASVEAAVGGTVTIKCQASQSISSYLAWYQQKPGQPPKLLIYKASTLASGVPSRFKGSGSGTEFTLTISDLECADAATYYCRCIYGDSYGAAFGGGTEVVVQ

SEQ ID NO: 61 - protein, 111 aa, synthetic construct
AIDMTQTPSPVSATVGGTVTISCQSSKSVVNGDWLAWYQQKPGQPPKLLIYDAATLASGVPSRFKGSGSGTQFTLTISDVQCADAATYYCAGVYNNDSDNGFGGGTEVVVK

SEQ ID NO: 62 - protein, 110 aa, synthetic construct
DIVLTQTAASVSEPVGGTVTIKCQASEYIYSSLAWYQQKPGQPPKLLIYDASDLASGVPSRFKGSGYGTEFTLTISGVQCGDAATYYCQCTDLSSSAGNTFGGGTEVVVK

SEQ ID NO: 63 - protein, 110 aa, synthetic construct
DVVMTQTASPVSAAVGGTVTINCQASEDIYTNLAWFQQKPGQPPKLLIYAASTLASGVPSRFSGSGSGTEFTLTISGLQCDDAATYFCLGVYTYISADGAFGGGTEVVVK

SEQ ID NO: 64 - protein, 330 aa, synthetic construct
ASTKGPSVFPLAPSSKSTSGGTAALGCLVKDYFPEPVTVSWNSGALTSGVHTFPAVLQSSGLYSLSSVVTVPSSSLGTQTYICNVNHKPSNTKVDKKVEPKSCDKTHTCPPCPAPELLGGPSVFLFPPKPKDTLMISRTPEVTCVVVDVSHEDPEVKFNWYVDGVEVHNAKTKPREEQYNSTYRVVSVLTVLHQDWLNGKEYKCKVSNKALPAPIEKTISKAKGQPREPQVYTLPPSREEMTKNQVSLTCLVKGFYPSDIAVEWESNGQPENNYKTTPPVLDSDGSFFLYSKLTVDKSRWQQGNVFSCSVMHEALHNHYTQKSLSLSPGK

SEQ ID NO: 65 - protein, 327 aa, synthetic construct
ASTKGPSVFPLAPCSRSTSESTAALGCLVKDYFPEPVTVSWNSGALTSGVHTFPAVLQSSGLYSLSSVVTVPSSSLGTKTYTCNVDHKPSNTKVDKRVESKYGPPCPSCPAPEFLGGPSVFLFPPKPKDTLMISRTPEVTCVVVDVSQEDPEVQFNWYVDGVEVHNAKTKPREEQFNSTYRVVSVLTVLHQDWLNGKEYKCKVSNKGLPSSIEKTISKAKGQPREPQVYTLPPSQEEMTKNQVSLTCLVKGFYPSDIAVEWESNGQPENNYKTTPPVLDSDGSFFLYSRLTVDKSRWQEGNVFSCSVMHEALHNHYTQKSLSLSLGK

SEQ ID NO: 66 - protein, 107 aa, synthetic construct [sequence omitted]

SEQ ID NO: 67 - protein, 106 aa, synthetic construct
GQPKAAPSVTLFPPSSEELQANKATLVCLISDFYPGAVTVAWKADSSPVKAGVETTTPSKQSNNKYAASSYLSLTPEQWKSHRSYSCQVTHEGSTVEKTVAPTECS

SEQ ID NO: 68 - protein, 308 aa, synthetic construct
MPGQELRTVNGSQMLLVLLVLSWLPHGGALSLAEASRASFPGPSELHSEDSRFRELRKRYEDLLTRLRANQSWEDSNTDLVPAPAVRILTPEVRLGSGGHLHLRISRAALPEGLPEASRLHRALFRLSPTASRSWDVTRPLRRQLSLARPQAPALHLRLSPPPSQSDQLLAESSSARPQLELHLRPQAARGRRRARARNGDHCPLGPGRCCRLHTVRASLEDLGWADWVLSPREVQVTMCIGACPSQFRAANMHAQIKTSLHRLKPDTVPAPCCVPASYNPMVLIQKTDTGVSLQTYDDLLAKDCHCI

SEQ ID NO: 69 - protein, 112 aa, synthetic construct
ARNGDHCPLGPGRCCRLHTVRASLEDLGWADWVLSPREVQVTMCIGACPSQFRAANMHAQIKTSLHRLKPDTVPAPCCVPASYNPMVLIQKTDTGVSLQTYDDLLAKDCHCI

SEQ ID NO: 70 - protein, 343 aa, synthetic construct
PCPAPELLGGPSVFLFPPKPKDTLMISRTPEVTCVVVDVSHEDPEVKFNWYVDGVEVHNAKTKPREEQYGSTYRVVSVLTVLHQDWLNGKEYKCKVSNKALPAPIEKTISKAKGQPREPQVYTLPPCRDELTKNQVSLWCLVKGFYPSDIAVEWESNGQPENNYKTTPPVLDSDGSFFLYSKLTVDKSRWQQGNVFSCSVMHEALHNHYTQKSLSLSPGENLYFQSGGGGSARNGDHCPLGPGRCCRLHTVRASLEDLGWADWVLSPREVQVTMCIGACPSQFRAANMHAQIKTSLHRLKPDTVPAPCCVPASYNPMVLIQKTDTGVSLQTYDDLLAKDCHCI

SEQ ID NO: 71 - protein, 343 aa, synthetic construct
PCPAPELLGGPSVFLFPPKPKDTLMISRTPEVTCVVVDVSHEDPEVKFNWYVDGVEVHNAKTKPREEQYGSTYRVVSVLTVLHQDWLNGKEYKCKVSNKALPAPIEKTISKAKGQPREPQVYTLPPCRDELTKNQVSLWCLVKGFYPSDIAVEWESNGQPENNYKTTPPVLDSDGSFFLYSKLTVDKSRWQQGNVFSCSVMHEALHNHYTQKSLSLSPGENLYFQSGGGGSARNGDRCPLGPGRCCRLHTVHASLEDLGWADWVLSPREVQVTMCIGACPSQFREANMHAQIKMNLHRLKPDTVPAPCCVPASYNPMVLIQKTDTGVSLQTYDDLLAKDCHCV

SEQ ID NO: 72 - protein, 343 aa, synthetic construct
PCPAPELLGGPSVFLFPPKPKDTLMISRTPEVTCVVVDVSHEDPEVKFNWYVDGVEVHNAKTKPREEQYGSTYRVVSVLTVLHQDWLNGKEYKCKVSNKALPAPIEKTISKAKGQPREPQVYTLPPCRDELTKNQVSLWCLVKGFYPSDIAVEWESNGQPENNYKTTPPVLDSDGSFFLYSKLTVDKSRWQQGNVFSCSVMHEALHNHYTQKSLSLSPGENLYFQSGGGGSAHPRDSCPLGPGRCCHLETVQATLEDLGWSDWVLSPRQLQLSMCVGECPHLYRSANTHAQIKARLHGLQPDKVPAPCCVPSSYTPVVLMHRTDSGVSLQTYDDLVARGCHCA

SEQ ID NO: 73 - protein, 233 aa, synthetic construct
MGHHHHHHGSLQASDSEVNQEAKPEVKPEVKPETHINLKVSDGSSEIFFKIKKTTPLRRLMEAFAKRQGKEMDSLRFLYDGIRIQADQAPEDLDMEDNDIIEAHREQIGGIEENLYFQSGSARNGDHCPLGPGRCCRLHTVRASLEDLGWADWVLSPREVQVTMCIGACPSQFRAANMHAQIKTSLHRLKPDTVPAPCCVPASYNPMVLIQKTDTGVSLQTYDDLLAKDCHCI

SEQ ID NO: 74 - protein, 344 aa, synthetic construct
SQTNNCTYLREQCLRDANGCKHAWRVMEDACNDSDPGDPCKMRNSSYCNLSIQYLVESNFQFKECLCTDDFYCTVNKLLGKKCINKSDNVKEDKFKWNLTTRSHHGFKGMWSCLEVAEACVGDVVCNAQLASYLKACSANGNPCDLKQCQAAIRFFYQNIPFNIAQMLAFCDCAQSDIPCQQSKEALHSKTCAVNMVPPPTCLSVIRSCQNDELCRRHYRTFQSKCWQRVTRKCHEDENCISTLSKQDLTCSGSDDCKAAYIDILGTVLQVQCTCRTITQSEESLCKIFQHMLHRKSCFNYPTLSNVKGMALYTRKHANKITLTGFHSPFNGEGGGGSHHHHHH

SEQ ID NO: 75 - protein, 16 aa, synthetic construct
IISGSGNTYYASWAKG

SEQ ID NO: 76 - protein, 16 aa, synthetic construct
IISSSGNTYYASWAKG

SEQ ID NO: 77 - protein, 16 aa, synthetic construct
IISNSGSTYYASWAKG

SEQ ID NO: 78 - protein, 16 aa, synthetic construct
IISGSGSTYYASWAKG

SEQ ID NO: 79 - protein, 16 aa, synthetic construct
  VARIANT 3: note = X is N or S
  VARIANT 4: note = X is G, N or S
  VARIANT 7: note = X is N or S
IIXXSGXTYYASWAKG

SEQ ID NO: 80 - protein, 12 aa, synthetic construct
LGVYTYISAEGA

SEQ ID NO: 81 - protein, 12 aa, synthetic construct
  VARIANT 10: note = X is D or E
LGVYTYISAXGA

SEQ ID NO: 82 - protein, 121 aa, synthetic construct
EVQLLESGGGLVQPGGSLRLSCAVSGFSLSSYDMTWVRQAPGKGLEWIGIISGSGNTYYASWAKGRFTISRDNSKNTVYLQMNSLRAEDTAVYFCARGILVYADYGDHNLWGQGTLVTVSS

SEQ ID NO: 83 - protein, 121 aa, synthetic construct
EVQLLESGGGLVQPGGSLRLSCAVSGFSLSSYDMTWVRQAPGKGLEWIGIISSSGNTYYASWAKGRFTISRDNSKNTVYLQMNSLRAEDTAVYFCARGILVYADYGDHNLWGQGTLVTVSS

SEQ ID NO: 84 - protein, 121 aa, synthetic construct
EVQLLESGGGLVQPGGSLRLSCAVSGFSLSSYDMTWVRQAPGKGLEWIGIISNSGSTYYASWAKGRFTISRDNSKNTVYLQMNSLRAEDTAVYFCARGILVYADYGDHNLWGQGTLVTVSS

SEQ ID NO: 85 - protein, 121 aa, synthetic construct
EVQLLESGGGLVQPGGSLRLSCAVSGFSLSSYDMTWVRQAPGKGLEWIGIISGSGSTYYASWAKGRFTISRDNSKNTVYLQMNSLRAEDTAVYFCARGILVYADYGDHNLWGQGTLVTVSS

SEQ ID NO: 86 - protein, 121 aa, synthetic construct
EVQLLESGGGLVQPGGSLRLSCAVSGFSLSSYDMTWVRQAPGKGLEWIGIISGSGNTYYASWAKGRFTISKDSSKNTVYLQMNSLRAEDTAVYFCARGILVYADYGDHNLWGQGTLVTVSS

SEQ ID NO: 87 - protein, 121 aa, synthetic construct
EVQLLESGGGLVQPGGSLRLSCAVSGFSLSSYDMTWVRQAPGKGLEWIGIISSSGNTYYASWAKGRFTISKDSSKNTVYLQMNSLRAEDTAVYFCARGILVYADYGDHNLWGQGTLVTVSS

SEQ ID NO: 88 - protein, 121 aa, synthetic construct
EVQLLESGGGLVQPGGSLRLSCAVSGFSLSSYDMTWVRQAPGKGLEWIGIISNSGSTYYASWAKGRFTISKDSSKNTVYLQMNSLRAEDTAVYFCARGILVYADYGDHNLWGQGTLVTVSS

SEQ ID NO: 89 - protein, 121 aa, synthetic construct
EVQLLESGGGLVQPGGSLRLSCAVSGFSLSSYDMTWVRQAPGKGLEWIGIISGSGSTYYASWAKGRFTISKDSSKNTVYLQMNSLRAEDTAVYFCARGILVYADYGDHNLWGQGTLVTVSS

SEQ ID NO: 90 - protein, 110 aa, synthetic construct
DIVMTQSPATLSVSPGERATLSCQASEDIYTNLAWFQQKPGQPPRLLIYAASTLASGIPARFSGSGSGTEFTLTISSLQSEDFAVYFCLGVYTYISAEGAFGQGTKVEIK

SEQ ID NO: 91 - protein, 110 aa, synthetic construct
DIVMTQSPATLSVSPGERATLSCQASEDIYTNLAWFQQKPGQPPRLLIYAASTLASGIPARFSGSGSGTEFTLTISSLQSEDFAVYYCLGVYTYISAEGAFGQGTKVEIK